European Patent Specification EP 3 436 607 B1, published June 14, 2023. Title: LINKED TARGET CAPTURE. Applicant: Boreal Genomics, Inc. Pel, Joel Marziali, Andrea. The sequence listing filed with the application follows.

SEQUENCE LISTING (4 sequences)

SEQ ID NO: 1 - DNA, 12 bp, Artificial Sequence
  Ligation Adapter Stem Region
cctactcgctac

SEQ ID NO: 2 - DNA, 12 bp, Artificial Sequence
  Ligation Adapter
atgcgagcctct

SEQ ID NO: 3 - DNA, 12 bp, Artificial Sequence
  Ligation Adapter Stem Region
gcacctcatcca

SEQ ID NO: 4 - DNA, 12 bp, Artificial Sequence
  Ligation Adapter Stem Region
tgcaggatggtg